European Patent Specification EP 3 464 374 B1, published August 6, 2025. Title: BAFF-R ANTIBODIES AND USES THEREOF. Applicant: Board of Regents, the University of Texas System City of Hope. The sequence listing filed with the application follows.

SEQUENCE LISTING (32 sequences)

SEQ ID NO: 1 - protein, 10 aa, mus musculus
ESVDNYGISF

SEQ ID NO: 2 - protein, 3 aa, mus musculus
AAS

SEQ ID NO: 3 - protein, 9 aa, mus musculus
QQSKEVPWT

SEQ ID NO: 4 - protein, 8 aa, mus musculus
GDSITSGY

SEQ ID NO: 5 - protein, 7 aa, mus muculus
ISYSGST

SEQ ID NO: 6 - protein, 12 aa, mus muculus
ASPNYPFYAMDY

SEQ ID NO: 7 - protein, 6 aa, mus muculus
QDISNY

SEQ ID NO: 8 - protein, 3 aa, mus muculus
YTS

SEQ ID NO: 9 - protein, 7 aa, mus muculus
FSELPWT

SEQ ID NO: 10 - protein, 10 aa, mus muculus
GFSLSTSGMG

SEQ ID NO: 11 - protein, 7 aa, mus muculus
IWWDDDK

SEQ ID NO: 12 - protein, 10 aa, mus muculus
ARSFGYGLDY

SEQ ID NO: 13 - DNA, 411 bp, artificial sequence
  synthetic construct
atgtacaggatgcaactcctgtcttgcattgcactaagtcttgcacttgtcacgaattcagacattgtgctgacccaatctccagcttctttggctgtgtctctagggcagagggccaccatctcctgcagagccagcgaaagtgttgataattatggcattagttttatgaactggttccaacagaaaccaggacagccacccaaactcctcatctatgctgcatccaaccaaggatccggggtccctgccaggtttagtggcagtgggtctgggacagacttcagcctcaacatccatcctatggaggaggatgatactgcaatgtatttctgtcagcaaagtaaggaggttccgtggacgttcggtggaggcaccaagctggaaatcaaaaccatggaaatcaaacgt

SEQ ID NO: 14 - protein, 137 aa, artificial sequence
  synthetic construct
MYRMQLLSCIALSLALVTNSDIVLTQSPASLAVSLGQRATISCRASESVDNYGISFMNWFQQKPGQPPKLLIYAASNQGSGVPARFSGSGSGTDFSLNIHPMEEDDTAMYFCQQSKEVPWTFGGGTKLEIKTMEIKR

SEQ ID NO: 15 - DNA, 420 bp, artificial sequence
  synthetic construct
atgtacaggatgcaactcctgtcttgcattgcactaagtcttgcacttgtcacgaattcggaggtgcagctgcaggagtctggacctagcctcgtgaaaccttctcagactctgtccctcacctgttctgtcactggcgactccatcaccagtggttactggaactggatccggaaattcccagggaataaacttgagtacatggggtacataagctacagtggtagcacttactacaatccatctctcaaaagtcgaatctccatcactcgagacacatccaagaaccagtactacctgcagttaaattctgtgacacctgaggacacagccacatattactgtgcaagccccaattaccccttctatgctatggactactggggtcaaggaacctcagtcaccgtctcctcagatatc

SEQ ID NO: 16 - protein, 140 aa, artificial sequence
  synthetic construct
MYRMQLLSCIALSLALVTNSEVQLQESGPSLVKPSQTLSLTCSVTGDSITSGYWNWIRKFPGNKLEYMGYISYSGSTYYNPSLKSRISITRDTSKNQYYLQLNSVTPEDTATYYCASPNYPFYAMDYWGQGTSVTVSSDI

SEQ ID NO: 17 - DNA, 403 bp, artificial sequence
  synthetic construct
atggagaccgacaccctgctgctctgggtgctgctgctctgggtgcccggctccaccggagagatcgtgctgacccagagccctgccaccctgtctctgagccctggcgagagagctaccctgtcctgcagagcctccgagtccgtggacaactacggcatctccttcctgaactggttccagcagaagcccggccaggcccccagactgctgatctacgccgcctctaatcgggccaccggcatccctgccagattctccggatctggctccggcaccgactttaccctgaccatctccagcctggaacccgaggacttcgccgtgtactactgccagcagtccaaagaggtgccctggacctttggcggaggcaccaaggtggaaatcaagcggaccgtgg

SEQ ID NO: 18 - protein, 134 aa, artificial sequence
  synthetic construct
METDTLLLWVLLLWVPGSTGEIVLTQSPATLSLSPGERATLSCRASESVDNYGISFLNWFQQKPGQAPRLLIYAASNRATGIPARFSGSGSGTDFTLTISSLEPEDFAVYYCQQSKEVPWTFGGGTKVEIKRTV

SEQ ID NO: 19 - DNA, 403 bp, artificial sequence
  synthetic construct
atggagaccgacaccctgctgctctgggtgctgctgctctgggtgcccggctccaccggagacatcgtgctgacccagagccctgccaccctgtctctgagccctggcgagagagctaccctgtcctgcagagcctccgagtccgtggacaactacggcatctccttcatgaactggttccagcagaagcccggccaggcccccagactgctgatctacgccgcctctaatcgggccaccggcatccctgccagattctccggatctggctccggcaccgactttaccctgaccatctccagcctggaacccgaggacttcgccgtgtactactgccagcagtccaaagaggtgccctggacctttggcggaggcaccaaggtggaaatcaagcggaccgtgg

SEQ ID NO: 20 - protein, 134 aa, artificial sequence
  synthetic construct
METDTLLLWVLLLWVPGSTGDIVLTQSPATLSLSPGERATLSCRASESVDNYGISFMNWFQQKPGQAPRLLIYAASNRATGIPARFSGSGSGTDFTLTISSLEPEDFAVYYCQQSKEVPWTFGGGTKVEIKRTV

SEQ ID NO: 21 - DNA, 403 bp, artificial sequence
  synthetic construct
atggagaccgacaccctgctgctctgggtgctgctgctctgggtgcccggctccaccggagacatcgtgatgacccagagcccctccagcctgtctgcctctgtgggcgacagagtgaccatcacctgtcgggcctccgagtccgtggacaactacggcatctccttcatgaactggttccagcagaagcccggcaaggcccccaagctgctgatctacgccgcctctaatctgggctctggcgtgccctctagattctccggatctggctccggcaccgactttaccctgaccatctccagcctgcagcccgaggacttcgccacctactactgccagcagtccaaagaggtgccctggacctttggccagggcaccaaggtggaaatcaagcggaccgtgg

SEQ ID NO: 22 - protein, 134 aa, artificial sequence
  synthetic construct
METDTLLLWVLLLWVPGSTGDIVMTQSPSSLSASVGDRVTITCRASESVDNYGISFMNWFQQKPGKAPKLLIYAASNLGSGVPSRFSGSGSGTDFTLTISSLQPEDFATYYCQQSKEVPWTFGQGTKVEIKRTV

SEQ ID NO: 23 - DNA, 426 bp, artificial sequence
  synthetic construct
atggaccccaagggcagcctgagctggagaatcctgctgttcctgagcctggccttcgagctgagctacggccaggtgcagctgcaggaatctggccctggcctcgtgaagccttcccagaccctgtccctgacctgcaccgtgtccggcgactctatcacctccggctactggaactggatccggcagcatcctggcaagggcctggagtatatcggctacatctcctactccggctccacctactacaaccccagcctgaagtccagagtgaccatctcccgggacacctccaagaaccagttctccctgaagctgtcctccgtgaccgctgctgataccgccgtgtactactgcgcctcccccaactaccccttctacgccatggactactggggccagggcaccctcgtgaccgtgtcctct

SEQ ID NO: 24 - protein, 142 aa, artificial sequence
  synthetic construct
MDPKGSLSWRILLFLSLAFELSYGQVQLQESGPGLVKPSQTLSLTCTVSGDSITSGYWNWIRQHPGKGLEYIGYISYSGSTYYNPSLKSRVTISRDTSKNQFSLKLSSVTAADTAVYYCASPNYPFYAMDYWGQGTLVTVSS

SEQ ID NO: 25 - DNA, 426 bp, artificial sequence
  synthetic construct
atggaccccaagggcagcctgagctggagaatcctgctgttcctgagcctggccttcgagctgagctacggcgaagtgcagctgcaggaatctggccctggcctcgtgaagccttcccagaccctgtccctgacctgcaccgtgtccggcgactctatcacctccggctactggaactggatccggcagcatcctggcaagggcctggagtatatcggctacatctcctactccggctccacctactacaaccccagcctgaagtccagagtgaccatctcccgggacacctccaagaaccagtactccctgaagctgtcctccgtgaccgctgctgataccgccgtgtactactgcgcctcccccaactaccccttctacgccatggactactggggccagggcaccctcgtgaccgtgtcctct

SEQ ID NO: 26 - protein, 142 aa, artificial sequence
  synthetic construct
MDPKGSLSWRILLFLSLAFELSYGEVQLQESGPGLVKPSQTLSLTCTVSGDSITSGYWNWIRQHPGKGLEYIGYISYSGSTYYNPSLKSRVTISRDTSKNQYSLKLSSVTAADTAVYYCASPNYPFYAMDYWGQGTLVTVSS

SEQ ID NO: 27 - DNA, 426 bp, artificial sequence
  synthetic construct
atggaccccaagggcagcctgagctggagaatcctgctgttcctgagcctggccttcgagctgagctacggcgaagtgcagctgcaggaatctggccctggcctcgtgaagccttccgagaccctgtccctgacctgctccgtgtccggcgactctatcacctccggctactggaactggatccggcagcctcctggcaagggcctggagtatatcggctacatctcctactccggctccacctactacaaccccagcctgaagtccagagtgaccatctcccgggacacctccaagaaccagtactccctgcggctgtcctccgtgaccgctgctgataccgccctgtactactgcgcctcccccaactaccccttctacgccatggactactggggccagggcacaagagtgaccgtgtcctct

SEQ ID NO: 28 - protein, 142 aa, artificial sequence
  synthetic construct
MDPKGSLSWRILLFLSLAFELSYGEVQLQESGPGLVKPSETLSLTCSVSGDSITSGYWNWIRQPPGKGLEYIGYISYSGSTYYNPSLKSRVTISRDTSKNQYSLRLSSVTAADTALYYCASPNYPFYAMDYWGQGTRVTVSS

SEQ ID NO: 29 - DNA, 387 bp, artificial sequence
  synthetic construct
atgtacaggatgcaactcctgtcttgcattgcactaagtcttgcacttgtcacgaattcagatatccagatgacacagactacatcctccctgtctgcctctctgggagacagagtcaccatcagttgcagtgcaagtcaggacattagcaattatttaaactggtatcagcagaaaccagatggaactgttaaactcctgatctattacacatcaagtttacactcaggagtcccatcaaggttcagtggcagtgggtctgggacagattattctctcaccatcagcagcctggaacctgaagatattgccacttactattgtcatcagtttagtgagcttccgtggacgttcggtggaggcaccaagctggaaataaaacgtacg

SEQ ID NO: 30 - protein, 129 aa, artificial sequence
  synthetic construct
MYRMQLLSCIALSLALVTNSDIQMTQTTSSLSASLGDRVTISCSASQDISNYLNWYQQKPDGTVKLLIYYTSSLHSGVPSRFSGSGSGTDYSLTISSLEPEDIATYYCHQFSELPWTFGGGTKLEIKRT

SEQ ID NO: 31 - DNA, 420 bp, artificial sequence
  synthetic construct
atgtacaggatgcaactcctgtcttgcattgcactaagtcttgcacttgtcacgaattcgcaggttactctgaaagagtctggccctgggatattgaagccctcacagaccctcagtctgacttgttctttctctgggttttcactgagcacttctggtatgggtgtaggctggattcgtcagccttcagggaagggtctggagtggctggcacacatttggtgggatgatgataaatactataactcatccctgaagagtcacctcacaatctccaaggatacctccagaaaccaggtattcctcaagatcaccagtgtggacactgcagatactgccacttactactgtgctcgaagctttggttacggtcttgactactggggccaaggcaccactctcacagtctcctcagctagc

SEQ ID NO: 32 - protein, 140 aa, artificial sequence
  synthetic construct
MYRMQLLSCIALSLALVTNSQVTLKESGPGILKPSQTLSLTCSFSGFSLSTSGMGVGWIRQPSGKGLEWLAHIWWDDDKYYNSSLKSHLTISKDTSRNQVFLKITSVDTADTATYYCARSFGYGLDYWGQGTTLTVSSAS